European Patent Application EP 4 563 700 A1, published June 4, 2025. Title: Novel acetohydroxy acid synthase small subunit variant and a method for producing L-valine using the same. Applicant: CJ CheilJedang Corporation. The sequence listing filed with the application follows.

SEQUENCE LISTING (12 sequences)

SEQ ID NO: 1 - protein, 172 aa, unidentified
MANSDVTRHILSVLVQDVDGIISRVSGMFTRRAFNLVSLVSAKTETLGINRITVVVDADELNIEQITKQLNKLIPVLKVVRLDEETTIARAIMLVKVSADSTNRPQIVDAANIFRARVVDVAPDSVVIESTGTPGKLRALLDVMEPFGIRELIQSGQIALNRGPKTMAPAKI

SEQ ID NO: 2 - DNA, 519 bp, unidentified
  source 1..519: mol_type = genomic DNA
atggctaattctgacgtcacccgccacatcctgtccgtactcgttcaggacgtagacggaatcatttcccgcgtatcaggtatgttcacccgacgcgcattcaacctcgtgtccctcgtgtctgcaaagaccgaaacactcggcatcaaccgcatcacggttgttgtcgacgccgacgagctcaacattgagcagatcaccaagcagctcaacaagctgatccccgtgctcaaagtcgtgcgacttgatgaagagaccaccatcgcccgcgcaatcatgctggttaaggtctctgcggatagcaccaaccgtccgcagatcgtcgacgccgcgaacatcttccgcgcccgagtcgtcgacgtggctccagactctgtggttattgaatccacaggcaccccaggcaagctccgcgcactgcttgatgtgatggaaccattcggaatccgcgaactgatccaatccggacagattgcactcaaccgcggtccgaagaccatggctccggccaagatctaa

SEQ ID NO: 3 - protein, 172 aa, synthetic construct
MANSDVTRHILSVLVQDVDGIISRVSGMFTRRAFNLVSLVSAKTETLGINRITVVVDADELNIEQITKQLNKLIPVLKVVRLDEETTIARAIMLVKVSADSTNRPQIVDAANIFRARVVDVAPDSVVIESTGTPGKLRALLDVMEPFGIRELIQSGQIELNRGPKTMAPAKI

SEQ ID NO: 4 - DNA, 519 bp, synthetic construct
  source 1..519: mol_type = other DNA
atggctaattctgacgtcacccgccacatcctgtccgtactcgttcaggacgtagacggaatcatttcccgcgtatcaggtatgttcacccgacgcgcattcaacctcgtgtccctcgtgtctgcaaagaccgaaacactcggcatcaaccgcatcacggttgttgtcgacgccgacgagctcaacattgagcagatcaccaagcagctcaacaagctgatccccgtgctcaaagtcgtgcgacttgatgaagagaccaccatcgcccgcgcaatcatgctggttaaggtctctgcggatagcaccaaccgtccgcagatcgtcgacgccgcgaacatcttccgcgcccgagtcgtcgacgtggctccagactctgtggttattgaatccacaggcaccccaggcaagctccgcgcactgcttgatgtgatggaaccattcggaatccgcgaactgatccaatccggacagattgaactcaaccgcggtccgaagaccatggctccggccaagatctaa

SEQ ID NO: 5 - protein, 172 aa, synthetic construct
MANSDVTRHILSVLVQDVDGIISRVSGMFTRRAFNLVSLVSVKTETLGINRITVVVDADELNIEQITKQLNKLIPVLKVVRLDEETTIARAIMLVKVSADSTNRPQIVDAANIFRARVVDVAPDSVVIESTGTPGKLRALLDVMEPFGIRELIQSGQIELNRGPKTMAPAKI

SEQ ID NO: 6 - DNA, 519 bp, synthetic construct
  source 1..519: mol_type = other DNA
atggctaattctgacgtcacccgccacatcctgtccgtactcgttcaggacgtagacggaatcatttcccgcgtatcaggtatgttcacccgacgcgcattcaacctcgtgtccctcgtgtctgtaaagaccgaaacactcggcatcaaccgcatcacggttgttgtcgacgccgacgagctcaacattgagcagatcaccaagcagctcaacaagctgatccccgtgctcaaagtcgtgcgacttgatgaagagaccaccatcgcccgcgcaatcatgctggttaaggtctctgcggatagcaccaaccgtccgcagatcgtcgacgccgcgaacatcttccgcgcccgagtcgtcgacgtggctccagactctgtggttattgaatccacaggcaccccaggcaagctccgcgcactgcttgatgtgatggaaccattcggaatccgcgaactgatccaatccggacagattgaactcaaccgcggtccgaagaccatggctccggccaagatctaa

SEQ ID NO: 7 - DNA, 41 bp, synthetic construct
  source 1..41: mol_type = other DNA
cggggatcctctagaaggacggtactcaaatactaaacttc

SEQ ID NO: 8 - DNA, 41 bp, synthetic construct
  source 1..41: mol_type = other DNA
cggggatcctctagagacaactacattattattataccaca

SEQ ID NO: 9 - DNA, 41 bp, synthetic construct; identical to SEQ ID NO: 7
  source 1..41: mol_type = other DNA

SEQ ID NO: 10 - DNA, 28 bp, synthetic construct
  source 1..28: mol_type = other DNA
ggtctttgcagacacgagggacacgagg

SEQ ID NO: 11 - DNA, 35 bp, synthetic construct
  source 1..35: mol_type = other DNA
tgtccctcgtgtctgcaaagaccgaaacactcggc

SEQ ID NO: 12 - DNA, 41 bp, synthetic construct; identical to SEQ ID NO: 8
  source 1..41: mol_type = other DNA